European Patent Specification EP 3 583 207 B1, published October 9, 2024. Title: NOVEL REVERSE TRANSCRIPTASES AND USES THEREOF. Applicant: Bio-Rad Laboratories, Inc. The sequence listing filed with the application follows.

SEQUENCE LISTING (42 sequences)

SEQ ID NO: 1 - protein, 222 aa, Artificial Sequence
  Synthetic construct
  MISC_FEATURE (140)..(140): Xaa = Leu or Pro
  MISC_FEATURE (201)..(201): Xaa = Asp or Asn
MTLNIEDEYRLHETSKEPDVSLGSTWLSDFPQAWAETGGMGLAVRQAPLIIPLKATSTPVSIKQYPMSQEARLGIKPHIQRLLDQGILVPCQSPWNTPLLPVKKPGTNDYRPVQDLREVNKRVEDIHPTVPNPYNLLSGXPPSHQWYTVLDLKDAFFCLRLHPTSQPLFAFEWRDPEMGISGQLTWTRLPQGFKNSPTLFXEALHRDLADFRIQHPDLILLQ

SEQ ID NO: 2 - protein, 278 aa, Artificial Sequence
  Synthetic construct
  MISC_FEATURE (140)..(140): Xaa = Leu or Pro
  MISC_FEATURE (201)..(201): Xaa = Asp or Asn
MTLNIEDEYRLHETSKEPDVSLGSTWLSDFPQAWAETGGMGLAVRQAPLIIPLKATSTPVSIKQYPMSQEARLGIKPHIQRLLDQGILVPCQSPWNTPLLPVKKPGTNDYRPVQDLREVNKRVEDIHPTVPNPYNLLSGXPPSHQWYTVLDLKDAFFCLRLHPTSQPLFAFEWRDPEMGISGQLTWTRLPQGFKNSPTLFXEALHRDLADFRIQHPDLILLQYVDDLLLAATSELDCQQGTRALLQTLGNLGYRASAKKAQICQKQVKYLGYLLKEGQ

SEQ ID NO: 3 - protein, 222 aa, Artificial Sequence
  Synthetic construct
MTLNIEDEYRLHETSKEPDVSLGSTWLSDFPQAWAETGGMGLAVRQAPLIIPLKATSTPVSIKQYPMSQEARLGIKPHIQRLLDQGILVPCQSPWNTPLLPVKKPGTNDYRPVQDLREVNKRVEDIHPTVPNPYNLLSGPPPSHQWYTVLDLKDAFFCLRLHPTSQPLFAFEWRDPEMGISGQLTWTRLPQGFKNSPTLFNEALHRDLADFRIQHPDLILLQ

SEQ ID NO: 4 - protein, 278 aa, Artificial Sequence
  Synthetic construct
MTLNIEDEYRLHETSKEPDVSLGSTWLSDFPQAWAETGGMGLAVRQAPLIIPLKATSTPVSIKQYPMSQEARLGIKPHIQRLLDQGILVPCQSPWNTPLLPVKKPGTNDYRPVQDLREVNKRVEDIHPTVPNPYNLLSGPPPSHQWYTVLDLKDAFFCLRLHPTSQPLFAFEWRDPEMGISGQLTWTRLPQGFKNSPTLFNEALHRDLADFRIQHPDLILLQYVDDLLLAATSELDCQQGTRALLQTLGNLGYRASAKKAQICQKQVKYLGYLLKEGQ

SEQ ID NO: 5 - protein, 391 aa, Artificial Sequence
  Synthetic construct
  MISC_FEATURE (245)..(245): Xaa = Asp, Gly, Asn, or Ala
  MISC_FEATURE (249)..(249): Xaa = Phe or Ile
  MISC_FEATURE (315)..(315): Xaa = His or Lys
  MISC_FEATURE (324)..(324): Xaa = Leu or Trp
  MISC_FEATURE (328)..(328): Xaa = Glu or Lys
  MISC_FEATURE (355)..(355): Xaa = His or Tyr
RWLTKARKEAILSIPVPKNPRQVREFLGTAGYCRLWIPGFAELAAPLYPLTRPGTLFQWGTEQQLAFENIRKALLSSPALGLPDITKPFELFIDENSGFAKGVLVQKLGPWKRPVAYLSKKLDTVASGWPPCLRMVAAIAILVKDAGKLTLGQPLTILTSHPVEALVRQPPNKWLSNARMTHYQAMLLDAERVHFGPTVSLNPATLLPLPSGKPPRLSPDLAETMAQTDLTDQPLPDADLTWYTXGSSXIRNGERKAGAAVTTESEVIWAASLPPGTSAQRAELIALTQALKMAKGKKLTVYTDSRYAFATAHVXGEIYRRRGXLTSXGKEIKNKNEILALLEALFLPKRLSIIXCPGHQKGDSPQAKGNRLADDTAKKAATETQSSLTIL

SEQ ID NO: 6 - protein, 406 aa, Artificial Sequence
  Synthetic construct
  MISC_FEATURE (245)..(245): Xaa = Asp, Gly, Asn, or Ala
  MISC_FEATURE (249)..(249): Xaa = Phe or Ile
  MISC_FEATURE (315)..(315): Xaa = His or Lys
  MISC_FEATURE (324)..(324): Xaa = Leu or Trp
  MISC_FEATURE (328)..(328): Xaa = Glu or Lys
  MISC_FEATURE (355)..(355): Xaa = His or Tyr
RWLTKARKEAILSIPVPKNPRQVREFLGTAGYCRLWIPGFAELAAPLYPLTRPGTLFQWGTEQQLAFENIRKALLSSPALGLPDITKPFELFIDENSGFAKGVLVQKLGPWKRPVAYLSKKLDTVASGWPPCLRMVAAIAILVKDAGKLTLGQPLTILTSHPVEALVRQPPNKWLSNARMTHYQAMLLDAERVHFGPTVSLNPATLLPLPSGKPPRLSPDLAETMAQTDLTDQPLPDADLTWYTXGSSXIRNGERKAGAAVTTESEVIWAASLPPGTSAQRAELIALTQALKMAKGKKLTVYTDSRYAFATAHVXGEIYRRRGXLTSXGKEIKNKNEILALLEALFLPKRLSIIXCPGHQKGDSPQAKGNRLADDTAKKAATETQSSLTILPTELIEGPKRPPWEY

SEQ ID NO: 7 - protein, 391 aa, Artificial Sequence
  Synthetic construct
RWLTKARKEAILSIPVPKNPRQVREFLGTAGYCRLWIPGFAELAAPLYPLTRPGTLFQWGTEQQLAFENIRKALLSSPALGLPDITKPFELFIDENSGFAKGVLVQKLGPWKRPVAYLSKKLDTVASGWPPCLRMVAAIAILVKDAGKLTLGQPLTILTSHPVEALVRQPPNKWLSNARMTHYQAMLLDAERVHFGPTVSLNPATLLPLPSGKPPRLSPDLAETMAQTDLTDQPLPDADLTWYTAGSSIIRNGERKAGAAVTTESEVIWAASLPPGTSAQRAELIALTQALKMAKGKKLTVYTDSRYAFATAHVHGEIYRRRGLLTSEGKEIKNKNEILALLEALFLPKRLSIIYCPGHQKGDSPQAKGNRLADDTAKKAATETQSSLTIL

SEQ ID NO: 8 - protein, 406 aa, Artificial Sequence
  Synthetic construct
RWLTKARKEAILSIPVPKNPRQVREFLGTAGYCRLWIPGFAELAAPLYPLTRPGTLFQWGTEQQLAFENIRKALLSSPALGLPDITKPFELFIDENSGFAKGVLVQKLGPWKRPVAYLSKKLDTVASGWPPCLRMVAAIAILVKDAGKLTLGQPLTILTSHPVEALVRQPPNKWLSNARMTHYQAMLLDAERVHFGPTVSLNPATLLPLPSGKPPRLSPDLAETMAQTDLTDQPLPDADLTWYTGGSSFIRNGERKAGAAVTTESEVIWAASLPPGTSAQRAELIALTQALKMAKGKKLTVYTDSRYAFATAHVHGEIYRRRGWLTSKGKEIKNKNEILALLEALFLPKRLSIIHCPGHQKGDSPQAKGNRLADDTAKKAATETQSSLTILPTELIEGPKRPPWEY

SEQ ID NO: 9 - protein, 391 aa, Artificial Sequence
  Synthetic construct
RWLTKARKEAILSIPVPKNPRQVREFLGTAGYCRLWIPGFAELAAPLYPLTRPGTLFQWGTEQQLAFENIRKALLSSPALGLPDITKPFELFIDENSGFAKGVLVQKLGPWKRPVAYLSKKLDTVASGWPPCLRMVAAIAILVKDAGKLTLGQPLTILTSHPVEALVRQPPNKWLSNARMTHYQAMLLDAERVHFGPTVSLNPATLLPLPSGKPPRLSPDLAETMAQTDLTDQPLPDADLTWYTGGSSFIRNGERKAGAAVTTESEVIWAASLPPGTSAQRAELIALTQALKMAKGKKLTVYTDSRYAFATAHVHGEIYRRRGWLTSKGKEIKNKNEILALLEALFLPKRLSIIHCPGHQKGDSPQAKGNRLADDTAKKAATETQSSLTIL

SEQ ID NO: 10 - protein, 447 aa, Artificial Sequence
  Synthetic construct
  MISC_FEATURE (301)..(301): Xaa = Asp, Gly, Asn, or Ala
  MISC_FEATURE (305)..(305): Xaa = Phe or Ile
  MISC_FEATURE (371)..(371): Xaa = His or Lys
  MISC_FEATURE (380)..(380): Xaa = Leu or Trp
  MISC_FEATURE (384)..(384): Xaa = Glu or Lys
  MISC_FEATURE (411)..(411): Xaa = His or Tyr
YVDDLLLAAATRTECLEGTKALLETLGNKGYRASAKKAQICLQEVTYLGYSLKDGQRWLTKARKEAILSIPVPKNPRQVREFLGTAGYCRLWIPGFAELAAPLYPLTRPGTLFQWGTEQQLAFENIRKALLSSPALGLPDITKPFELFIDENSGFAKGVLVQKLGPWKRPVAYLSKKLDTVASGWPPCLRMVAAIAILVKDAGKLTLGQPLTILTSHPVEALVRQPPNKWLSNARMTHYQAMLLDAERVHFGPTVSLNPATLLPLPSGKPPRLSPDLAETMAQTDLTDQPLPDADLTWYTXGSSXIRNGERKAGAAVTTESEVIWAASLPPGTSAQRAELIALTQALKMAKGKKLTVYTDSRYAFATAHVXGEIYRRRGXLTSXGKEIKNKNEILALLEALFLPKRLSIIXCPGHQKGDSPQAKGNRLADDTAKKAATETQSSLTIL

SEQ ID NO: 11 - protein, 447 aa, Artificial Sequence
  Synthetic construct
YVDDLLLAAATRTECLEGTKALLETLGNKGYRASAKKAQICLQEVTYLGYSLKDGQRWLTKARKEAILSIPVPKNPRQVREFLGTAGYCRLWIPGFAELAAPLYPLTRPGTLFQWGTEQQLAFENIRKALLSSPALGLPDITKPFELFIDENSGFAKGVLVQKLGPWKRPVAYLSKKLDTVASGWPPCLRMVAAIAILVKDAGKLTLGQPLTILTSHPVEALVRQPPNKWLSNARMTHYQAMLLDAERVHFGPTVSLNPATLLPLPSGKPPRLSPDLAETMAQTDLTDQPLPDADLTWYTGGSSFIRNGERKAGAAVTTESEVIWAASLPPGTSAQRAELIALTQALKMAKGKKLTVYTDSRYAFATAHVHGEIYRRRGWLTSKGKEIKNKNEILALLEALFLPKRLSIIHCPGHQKGDSPQAKGNRLADDTAKKAATETQSSLTIL

SEQ ID NO: 12 - protein, 447 aa, Artificial Sequence
  Synthetic construct
YVDDLLLAAATRTECLEGTKALLETLGNKGYRASAKKAQICLQEVTYLGYSLKDGQRWLTKARKEAILSIPVPKNPRQVREFLGTAGYCRLWIPGFAELAAPLYPLTRPGTLFQWGTEQQLAFENIRKALLSSPALGLPDITKPFELFIDENSGFAKGVLVQKLGPWKRPVAYLSKKLDTVASGWPPCLRMVAAIAILVKDAGKLTLGQPLTILTSHPVEALVRQPPNKWLSNARMTHYQAMLLDAERVHFGPTVSLDPATLLPLPSGKPPRLSPDLAETMAQTDLTDQPLPDADLTWYTDGSSFIRNGERKAGAAVTTESEVIWAASLPPGTSAQRAELIALTQALKMAKGKKLTVYTDSRYAFATAHVKGEIYRRRGWLTSEGKEIKNKNEILALLEALFLPKRLSIIHCPGHQKGDSPQAKGNRLADDTAKKAATETQSSLTIL

SEQ ID NO: 13 - protein, 447 aa, Artificial Sequence
  Synthetic construct
YVDDLLLAAATRTECLEGTKALLETLGNKGYRASAKKAQICLQEVTYLGYSLKDGQRWLTKARKEAILSIPVPKNPRQVREFLGTAGYCRLWIPGFAELAAPLYPLTRPGTLFQWGTEQQLAFENIRKALLSSPALGLPDITKPFELFIDENSGFAKGVLVQKLGPWKRPVAYLSKKLDTVASGWPPCLRMVAAIAILVKDAGKLTLGQPLTILTSHPVEALVRQPPNKWLSNARMTHYQAMLLDAERVHFGPTVSLNPATLLPLPSGKPPRLSPDLAETMAQTDLTDQPLPDADLTWYTGGSSFIRNGERKAGAAVTTESEVIWAASLPPGTSAQRAELIALTQALKMAKGKKLTVYTDSRYAFATAHVHGEIYRRRGWLTSEGKEIKNKNEILALLEALFLPKRLSIIHCPGHQKGDSPQAKGNRLANDTAKKAATETQSSLTIL

SEQ ID NO: 14 - protein, 669 aa, Artificial Sequence
  Synthetic construct
MTLNIEDEYRLHETSKEPDVSLGSTWLSDFPQAWAETGGMGLAVRQAPLIIPLKATSTPVSIKQYPMSQEARLGIKPHIQRLLDQGILVPCQSPWNTPLLPVKKPGTNDYRPVQDLREVNKRVEDIHPTVPNPYNLLSGPPPSHQWYTVLDLKDAFFCLRLHPTSQPLFAFEWRDPEMGISGQLTWTRLPQGFKNSPTLFNEALHRDLADFRIQHPDLILLQYVDDLLLAATSELDCQQGTRALLQTLGNLGYRASAKKAQICQKQVKYLGYLLKEGQRWLTKARKEAILSIPVPKNPRQVREFLGTAGYCRLWIPGFAELAAPLYPLTRPGTLFQWGTEQQLAFENIRKALLSSPALGLPDITKPFELFIDENSGFAKGVLVQKLGPWKRPVAYLSKKLDTVASGWPPCLRMVAAIAILVKDAGKLTLGQPLTILTSHPVEALVRQPPNKWLSNARMTHYQAMLLDAERVHFGPTVSLNPATLLPLPSGKPPRLSPDLAETMAQTDLTDQPLPDADLTWYTAGSSIIRNGERKAGAAVTTESEVIWAASLPPGTSAQRAELIALTQALKMAKGKKLTVYTDSRYAFATAHVHGEIYRRRGLLTSEGKEIKNKNEILALLEALFLPKRLSIIYCPGHQKGDSPQAKGNRLADDTAKKAATETQSSLTIL

SEQ ID NO: 15 - protein, 684 aa, Artificial Sequence
  Synthetic construct
MTLNIEDEYRLHETSKEPDVSLGSTWLSDFPQAWAETGGMGLAVRQAPLIIPLKATSTPVSIKQYPMSQEARLGIKPHIQRLLDQGILVPCQSPWNTPLLPVKKPGTNDYRPVQDLREVNKRVEDIHPTVPNPYNLLSGPPPSHQWYTVLDLKDAFFCLRLHPTSQPLFAFEWRDPEMGISGQLTWTRLPQGFKNSPTLFNEALHRDLADFRIQHPDLILLQYVDDLLLAATSELDCQQGTRALLQTLGNLGYRASAKKAQICQKQVKYLGYLLKEGQRWLTKARKEAILSIPVPKNPRQVREFLGTAGYCRLWIPGFAELAAPLYPLTRPGTLFQWGTEQQLAFENIRKALLSSPALGLPDITKPFELFIDENSGFAKGVLVQKLGPWKRPVAYLSKKLDTVASGWPPCLRMVAAIAILVKDAGKLTLGQPLTILTSHPVEALVRQPPNKWLSNARMTHYQAMLLDAERVHFGPTVSLNPATLLPLPSGKPPRLSPDLAETMAQTDLTDQPLPDADLTWYTGGSSFIRNGERKAGAAVTTESEVIWAASLPPGTSAQRAELIALTQALKMAKGKKLTVYTDSRYAFATAHVHGEIYRRRGWLTSKGKEIKNKNEILALLEALFLPKRLSIIHCPGHQKGDSPQAKGNRLADDTAKKAATETQSSLTILPTELIEGPKRPPWEY

SEQ ID NO: 16 - protein, 669 aa, Artificial Sequence
  Synthetic construct
MTLNIEDEYRLHETSKEPDVSLGSTWLSDFPQAWAETGGMGLAVRQAPLIIPLKATSTPVSIKQYPMSQEARLGIKPHIQRLLDQGILVPCQSPWNTPLLPVKKPGTNDYRPVQDLREVNKRVEDIHPTVPNPYNLLSGPPPSHQWYTVLDLKDAFFCLRLHPTSQPLFAFEWRDPEMGISGQLTWTRLPQGFKNSPTLFNEALHRDLADFRIQHPDLILLQYVDDLLLAATSELDCQQGTRALLQTLGNLGYRASAKKAQICQKQVKYLGYLLKEGQRWLTKARKEAILSIPVPKNPRQVREFLGTAGYCRLWIPGFAELAAPLYPLTRPGTLFQWGTEQQLAFENIRKALLSSPALGLPDITKPFELFIDENSGFAKGVLVQKLGPWKRPVAYLSKKLDTVASGWPPCLRMVAAIAILVKDAGKLTLGQPLTILTSHPVEALVRQPPNKWLSNARMTHYQAMLLDAERVHFGPTVSLNPATLLPLPSGKPPRLSPDLAETMAQTDLTDQPLPDADLTWYTGGSSFIRNGERKAGAAVTTESEVIWAASLPPGTSAQRAELIALTQALKMAKGKKLTVYTDSRYAFATAHVHGEIYRRRGWLTSKGKEIKNKNEILALLEALFLPKRLSIIHCPGHQKGDSPQAKGNRLADDTAKKAATETQSSLTIL

SEQ ID NO: 17 - protein, 669 aa, Artificial Sequence
  Synthetic construct
MTLNIEDEYRLHETSKEPDVSLGSTWLSDFPQAWAETGGMGLAVRQAPLIIPLKATSTPVSIKQYPMSQEARLGIKPHIQRLLDQGILVPCQSPWNTPLLPVKKPGTNDYRPVQDLREVNKRVEDIHPTVPNPYNLLSGPPPSHQWYTVLDLKDAFFCLRLHPTSQPLFAFEWRDPEMGISGQLTWTRLPQGFKNSPTLFNEALHRDLADFRIQHPDLILLQYVDDLLLAAATRTECLEGTKALLETLGNKGYRASAKKAQICLQEVTYLGYSLKDGQRWLTKARKEAILSIPVPKNPRQVREFLGTAGYCRLWIPGFAELAAPLYPLTRPGTLFQWGTEQQLAFENIRKALLSSPALGLPDITKPFELFIDENSGFAKGVLVQKLGPWKRPVAYLSKKLDTVASGWPPCLRMVAAIAILVKDAGKLTLGQPLTILTSHPVEALVRQPPNKWLSNARMTHYQAMLLDAERVHFGPTVSLNPATLLPLPSGKPPRLSPDLAETMAQTDLTDQPLPDADLTWYTGGSSFIRNGERKAGAAVTTESEVIWAASLPPGTSAQRAELIALTQALKMAKGKKLTVYTDSRYAFATAHVHGEIYRRRGWLTSKGKEIKNKNEILALLEALFLPKRLSIIHCPGHQKGDSPQAKGNRLADDTAKKAATETQSSLTIL

SEQ ID NO: 18 - protein, 669 aa, Artificial Sequence
  Synthetic construct
MTLNIEDEYRLHETSKEPDVSLGSTWLSDFPQAWAETGGMGLAVRQAPLIIPLKATSTPVSIKQYPMSQEARLGIKPHIQRLLDQGILVPCQSPWNTPLLPVKKPGTNDYRPVQDLREVNKRVEDIHPTVPNPYNLLSGLPPSHQWYTVLDLKDAFFCLRLHPTSQPLFAFEWRDPEMGISGQLTWTRLPQGFKNSPTLFNEALHRDLADFRIQHPDLILLQYVDDLLLAAATRTECLEGTKALLETLGNKGYRASAKKAQICLQEVTYLGYSLKDGQRWLTKARKEAILSIPVPKNPRQVREFLGTAGYCRLWIPGFAELAAPLYPLTRPGTLFQWGTEQQLAFENIRKALLSSPALGLPDITKPFELFIDENSGFAKGVLVQKLGPWKRPVAYLSKKLDTVASGWPPCLRMVAAIAILVKDAGKLTLGQPLTILTSHPVEALVRQPPNKWLSNARMTHYQAMLLDAERVHFGPTVSLDPATLLPLPSGKPPRLSPDLAETMAQTDLTDQPLPDADLTWYTDGSSFIRNGERKAGAAVTTESEVIWAASLPPGTSAQRAELIALTQALKMAKGKKLTVYTDSRYAFATAHVKGEIYRRRGWLTSEGKEIKNKNEILALLEALFLPKRLSIIHCPGHQKGDSPQAKGNRLADDTAKKAATETQSSLTIL

SEQ ID NO: 19 - protein, 447 aa, Artificial Sequence; identical to SEQ ID NO: 13
  Synthetic construct

SEQ ID NO: 20 - protein, 692 aa, Artificial Sequence
  Synthetic construct
MGSSHHHHHHSSGLVPRGSHMTLNIEDEYRLHETSKEPDVSLGSTWLSDFPQAWAETGGMGLAVRQAPLIIPLKATSTPVSIKQYPMSQEARLGIKPHIQRLLDQGILVPCQSPWNTPLLPVKKPGTNDYRPVQDLREVNKRVEDIHPTVPNPYNLLSGPPPSHQWYTVLDLKDAFFCLRLHPTSQPLFAFEWRDPEMGISGQLTWTRLPQGFKNSPTLFNEALHRDLADFRIQHPDLILLQYVDDLLLAATSELDCQQGTRALLQTLGNLGYRASAKKAQICQKQVKYLGYLLKEGQRWLTKARKEAILSIPVPKNPRQVREFLGTAGYCRLWIPGFAELAAPLYPLTRPGTLFQWGTEQQLAFENIRKALLSSPALGLPDITKPFELFIDENSGFAKGVLVQKLGPWKRPVAYLSKKLDTVASGWPPCLRMVAAIAILVKDAGKLTLGQPLTILTSHPVEALVRQPPNKWLSNARMTHYQAMLLDAERVHFGPTVSLNPATLLPLPSGKPPRLSPDLAETMAQTDLTDQPLPDADLTWYTAGSSIIRNGERKAGAAVTTESEVIWAASLPPGTSAQRAELIALTQALKMAKGKKLTVYTDSRYAFATAHVHGEIYRRRGLLTSEGKEIKNKNEILALLEALFLPKRLSIIYCPGHQKGDSPQAKGNRLADDTAKKAATETQSSLTILAAA

SEQ ID NO: 21 - protein, 707 aa, Artificial Sequence
  Synthetic construct
MGSSHHHHHHSSGLVPRGSHMTLNIEDEYRLHETSKEPDVSLGSTWLSDFPQAWAETGGMGLAVRQAPLIIPLKATSTPVSIKQYPMSQEARLGIKPHIQRLLDQGILVPCQSPWNTPLLPVKKPGTNDYRPVQDLREVNKRVEDIHPTVPNPYNLLSGPPPSHQWYTVLDLKDAFFCLRLHPTSQPLFAFEWRDPEMGISGQLTWTRLPQGFKNSPTLFNEALHRDLADFRIQHPDLILLQYVDDLLLAATSELDCQQGTRALLQTLGNLGYRASAKKAQICQKQVKYLGYLLKEGQRWLTKARKEAILSIPVPKNPRQVREFLGTAGYCRLWIPGFAELAAPLYPLTRPGTLFQWGTEQQLAFENIRKALLSSPALGLPDITKPFELFIDENSGFAKGVLVQKLGPWKRPVAYLSKKLDTVASGWPPCLRMVAAIAILVKDAGKLTLGQPLTILTSHPVEALVRQPPNKWLSNARMTHYQAMLLDAERVHFGPTVSLNPATLLPLPSGKPPRLSPDLAETMAQTDLTDQPLPDADLTWYTGGSSFIRNGERKAGAAVTTESEVIWAASLPPGTSAQRAELIALTQALKMAKGKKLTVYTDSRYAFATAHVHGEIYRRRGWLTSKGKEIKNKNEILALLEALFLPKRLSIIHCPGHQKGDSPQAKGNRLADDTAKKAATETQSSLTILPTELIEGPKRPPWEYAAA

SEQ ID NO: 22 - protein, 692 aa, Artificial Sequence
  Synthetic construct
MGSSHHHHHHSSGLVPRGSHMTLNIEDEYRLHETSKEPDVSLGSTWLSDFPQAWAETGGMGLAVRQAPLIIPLKATSTPVSIKQYPMSQEARLGIKPHIQRLLDQGILVPCQSPWNTPLLPVKKPGTNDYRPVQDLREVNKRVEDIHPTVPNPYNLLSGPPPSHQWYTVLDLKDAFFCLRLHPTSQPLFAFEWRDPEMGISGQLTWTRLPQGFKNSPTLFNEALHRDLADFRIQHPDLILLQYVDDLLLAATSELDCQQGTRALLQTLGNLGYRASAKKAQICQKQVKYLGYLLKEGQRWLTKARKEAILSIPVPKNPRQVREFLGTAGYCRLWIPGFAELAAPLYPLTRPGTLFQWGTEQQLAFENIRKALLSSPALGLPDITKPFELFIDENSGFAKGVLVQKLGPWKRPVAYLSKKLDTVASGWPPCLRMVAAIAILVKDAGKLTLGQPLTILTSHPVEALVRQPPNKWLSNARMTHYQAMLLDAERVHFGPTVSLNPATLLPLPSGKPPRLSPDLAETMAQTDLTDQPLPDADLTWYTGGSSFIRNGERKAGAAVTTESEVIWAASLPPGTSAQRAELIALTQALKMAKGKKLTVYTDSRYAFATAHVHGEIYRRRGWLTSKGKEIKNKNEILALLEALFLPKRLSIIHCPGHQKGDSPQAKGNRLADDTAKKAATETQSSLTILAAA

SEQ ID NO: 23 - protein, 692 aa, Artificial Sequence
  Synthetic construct
MGSSHHHHHHSSGLVPRGSHMTLNIEDEYRLHETSKEPDVSLGSTWLSDFPQAWAETGGMGLAVRQAPLIIPLKATSTPVSIKQYPMSQEARLGIKPHIQRLLDQGILVPCQSPWNTPLLPVKKPGTNDYRPVQDLREVNKRVEDIHPTVPNPYNLLSGPPPSHQWYTVLDLKDAFFCLRLHPTSQPLFAFEWRDPEMGISGQLTWTRLPQGFKNSPTLFNEALHRDLADFRIQHPDLILLQYVDDLLLAAATRTECLEGTKALLETLGNKGYRASAKKAQICLQEVTYLGYSLKDGQRWLTKARKEAILSIPVPKNPRQVREFLGTAGYCRLWIPGFAELAAPLYPLTRPGTLFQWGTEQQLAFENIRKALLSSPALGLPDITKPFELFIDENSGFAKGVLVQKLGPWKRPVAYLSKKLDTVASGWPPCLRMVAAIAILVKDAGKLTLGQPLTILTSHPVEALVRQPPNKWLSNARMTHYQAMLLDAERVHFGPTVSLNPATLLPLPSGKPPRLSPDLAETMAQTDLTDQPLPDADLTWYTGGSSFIRNGERKAGAAVTTESEVIWAASLPPGTSAQRAELIALTQALKMAKGKKLTVYTDSRYAFATAHVHGEIYRRRGWLTSKGKEIKNKNEILALLEALFLPKRLSIIHCPGHQKGDSPQAKGNRLADDTAKKAATETQSSLTILAAA

SEQ ID NO: 24 - protein, 692 aa, Artificial Sequence
  Synthetic construct
MGSSHHHHHHSSGLVPRGSHMTLNIEDEYRLHETSKEPDVSLGSTWLSDFPQAWAETGGMGLAVRQAPLIIPLKATSTPVSIKQYPMSQEARLGIKPHIQRLLDQGILVPCQSPWNTPLLPVKKPGTNDYRPVQDLREVNKRVEDIHPTVPNPYNLLSGLPPSHQWYTVLDLKDAFFCLRLHPTSQPLFAFEWRDPEMGISGQLTWTRLPQGFKNSPTLFNEALHRDLADFRIQHPDLILLQYVDDLLLAAATRTECLEGTKALLETLGNKGYRASAKKAQICLQEVTYLGYSLKDGQRWLTKARKEAILSIPVPKNPRQVREFLGTAGYCRLWIPGFAELAAPLYPLTRPGTLFQWGTEQQLAFENIRKALLSSPALGLPDITKPFELFIDENSGFAKGVLVQKLGPWKRPVAYLSKKLDTVASGWPPCLRMVAAIAILVKDAGKLTLGQPLTILTSHPVEALVRQPPNKWLSNARMTHYQAMLLDAERVHFGPTVSLDPATLLPLPSGKPPRLSPDLAETMAQTDLTDQPLPDADLTWYTDGSSFIRNGERKAGAAVTTESEVIWAASLPPGTSAQRAELIALTQALKMAKGKKLTVYTDSRYAFATAHVKGEIYRRRGWLTSEGKEIKNKNEILALLEALFLPKRLSIIHCPGHQKGDSPQAKGNRLADDTAKKAATETQSSLTILAAA

SEQ ID NO: 25 - protein, 692 aa, Artificial Sequence
  Synthetic construct
MGSSHHHHHHSSGLVPRGSHMTLNIEDEYRLHETSKEPDVSLGSTWLSDFPQAWAETGGMGLAVRQAPLIIPLKATSTPVSIKQYPMSQEARLGIKPHIQRLLDQGILVPCQSPWNTPLLPVKKPGTNDYRPVQDLREVNKRVEDIHPTVPNPYNLLSGLPPSHQWYTVLDLKDAFFCLRLHPTSQPLFAFEWRDPEMGISGQLTWTRLPQGFKNSPTLFNEALHRDLADFRIQHPDLILLQYVDDLLLAAATRTECLEGTKALLETLGNKGYRASAKKAQICLQEVTYLGYSLKDGQRWLTKARKEAILSIPVPKNPRQVREFLGTAGYCRLWIPGFAELAAPLYPLTRPGTLFQWGTEQQLAFENIRKALLSSPALGLPDITKPFELFIDENSGFAKGVLVQKLGPWKRPVAYLSKKLDTVASGWPPCLRMVAAIAILVKDAGKLTLGQPLTILTSHPVEALVRQPPNKWLSNARMTHYQAMLLDAERVHFGPTVSLNPATLLPLPSGKPPRLSPDLAETMAQTDLTDQPLPDADLTWYTGGSSFIRNGERKAGAAVTTESEVIWAASLPPGTSAQRAELIALTQALKMAKGKKLTVYTDSRYAFATAHVHGEIYRRRGWLTSEGKEIKNKNEILALLEALFLPKRLSIIHCPGHQKGDSPQAKGNRLANDTAKKAATETQSSLTILAAA

SEQ ID NO: 26 - protein, 279 aa, Unknown
  Feline Leukemia Virus
MTLQLEEEYRLFEPESTQKQEMDIWLKNFPQAWAETGGMGMAHCQAPVLIQLKATATPISIRQYPMPHEAYQGIKPHIRRMLDQGILKPCQSPWNTPLLPVKKPGTKDYRPVQDLREVNKRVEDIHPTVPNPYNLLSTLPPSHPWYTVLDLKDAFFCLRLHSESQLLFAFEWRDPEIGLSGQLTWTRLPQGFKNSPTLFDEALHSDLADFRVRYPALVLLQYVDDLLLAAATRTECLEGTKALLETLGNKGYRASAKKAQICLQEVTYLGYSLKDGQRW

SEQ ID NO: 27 - protein, 497 aa, Unknown
  Feline Leukemia Virus
MTLQLEEEYRLFEPESTQKQEMDIWLKNFPQAWAETGGMGMAHCQAPVLIQLKATATPISIRQYPMPHEAYQGIKPHIRRMLDQGILKPCQSPWNTPLLPVKKPGTKDYRPVQDLREVNKRVEDIHPTVPNPYNLLSTLPPSHPWYTVLDLKDAFFCLRLHSESQLLFAFEWRDPEIGLSGQLTWTRLPQGFKNSPTLFDEALHSDLADFRVRYPALVLLQYVDDLLLAAATRTECLEGTKALLETLGNKGYRASAKKAQICLQEVTYLGYSLKDGQRWLTKARKEAILSIPVPKNPRQVREFLGTAGYCRLWIPGFAELAAPLYPLTRPGTLFQWGTEQQLAFENIRKALLSSPALGLPDITKPFELFIDENSGFAKGVLVQKLGPWKRPVAYLSKKLDTVASGWPPCLRMVAAIAILVKDAGKLTLGQPLTILTSHPVEALVRQPPNKWLSNARMTHYQAMLLDAERVHFGPTVSLNPATLLPLPSGKPPRLSPD

SEQ ID NO: 28 - protein, 392 aa, Unknown
  Mouse Leukemia Virus
LTEARKETVMGQPTPKTPRQLREFLGTAGFCRLWIPGFAEMAAPLYPLTKTGTLFNWGPDQQKAYQEIKQALLTAPALGLPDLTKPFELFVDEKQGYAKGVLTQKLGPWRRPVAYLSKKLDPVAAGWPPCLRMVAAIAVLTKDAGKLTMGQPLVILAPHAVEALVKQPPDRWLSNARMTHYQALLLDTDRVQFGPVVALNPATLLPLPEEGLQHDCLDILAEAHGTRSDLTDQPLPDADHTWYTDGSSFLQEGQRKAGAAVTTETEVIWARALPAGTSAQRAELIALTQALKMAEGKKLNVYTDSRYAFATAHIHGEIYRRRGLLTSEGKEIKNKDEILALLKALFLPKRLSIIHCPGHQKGNSAEARGNRMADQAAREVATRETPGTSTLL

SEQ ID NO: 29 - protein, 174 aa, Unknown
  Mouse Leukemia Virus
ILAEAHGTRSDLTDQPLPDADHTWYTDGSSFLQEGQRKAGAAVTTETEVIWARALPAGTSAQRAELIALTQALKMAEGKKLNVYTDSRYAFATAHIHGEIYRRRGLLTSEGKEIKNKDEILALLKALFLPKRLSIIHCPGHQKGNSAEARGNRMADQAAREVATRETPGTSTLL

SEQ ID NO: 30 - protein, 671 aa, Artificial Sequence
  Synthetic construct
MTLQLEEEYRLFEPESTQKQEMDIWLKNFPQAWAETGGMGMAHCQAPVLIQLKATATPISIRQYPMPHEAYQGIKPHIRRMLDQGILKPCQSPWNTPLLPVKKPGTKDYRPVQDLREVNKRVEDIHPTVPNPYNLLSTLPPSHPWYTVLDLKDAFFCLRLHSESQLLFAFEWRDPEIGLSGQLTWTRLPQGFKNSPTLFDEALHSDLADFRVRYPALVLLQYVDDLLLAAATRTECLEGTKALLETLGNKGYRASAKKAQICLQEVTYLGYSLKDGQRWLTEARKETVMGQPTPKTPRQLREFLGTAGFCRLWIPGFAEMAAPLYPLTKTGTLFNWGPDQQKAYQEIKQALLTAPALGLPDLTKPFELFVDEKQGYAKGVLTQKLGPWRRPVAYLSKKLDPVAAGWPPCLRMVAAIAVLTKDAGKLTMGQPLVILAPHAVEALVKQPPDRWLSNARMTHYQALLLDTDRVQFGPVVALNPATLLPLPEEGLQHDCLDILAEAHGTRSDLTDQPLPDADHTWYTDGSSFLQEGQRKAGAAVTTETEVIWARALPAGTSAQRAELIALTQALKMAEGKKLNVYTDSRYAFATAHIHGEIYRRRGLLTSEGKEIKNKDEILALLKALFLPKRLSIIHCPGHQKGNSAEARGNRMADQAAREVATRETPGTSTLL

SEQ ID NO: 31 - protein, 671 aa, Artificial Sequence
  Synthetic construct
MTLQLEEEYRLFEPESTQKQEMDIWLKNFPQAWAETGGMGMAHCQAPVLIQLKATATPISIRQYPMPHEAYQGIKPHIRRMLDQGILKPCQSPWNTPLLPVKKPGTKDYRPVQDLREVNKRVEDIHPTVPNPYNLLSTLPPSHPWYTVLDLKDAFFCLRLHSESQLLFAFEWRDPEIGLSGQLTWTRLPQGFKNSPTLFDEALHSDLADFRVRYPALVLLQYVDDLLLAAATRTECLEGTKALLETLGNKGYRASAKKAQICLQEVTYLGYSLKDGQRWLTKARKEAILSIPVPKNPRQVREFLGTAGYCRLWIPGFAELAAPLYPLTRPGTLFQWGTEQQLAFENIRKALLSSPALGLPDITKPFELFIDENSGFAKGVLVQKLGPWKRPVAYLSKKLDTVASGWPPCLRMVAAIAILVKDAGKLTLGQPLTILTSHPVEALVRQPPNKWLSNARMTHYQAMLLDAERVHFGPTVSLNPATLLPLPSGKPPRLSPDILAEAHGTRSDLTDQPLPDADHTWYTDGSSFLQEGQRKAGAAVTTETEVIWARALPAGTSAQRAELIALTQALKMAEGKKLNVYTDSRYAFATAHIHGEIYRRRGLLTSEGKEIKNKDEILALLKALFLPKRLSIIHCPGHQKGNSAEARGNRMADQAAREVATRETPGTSTLL

SEQ ID NO: 32 - protein, 671 aa, Unknown
  Mouse Leukemia Virus
TLNIEDEHRLHETSKEPDVSLGSTWLSDFPQAWAETGGMGLAVRQAPLIIPLKATSTPVSIKQYPMSQEARLGIKPHIQRLLDQGILVPCQSPWNTPLLPVKKPGTNDYRPVQDLREVNKRVEDIHPTVPNPYNLLSGLPPSHQWYTVLDLKDAFFCLRLHPTSQPLFAFEWRDPEMGISGQLTWTRLPQGFKNSPTLFDEALHRDLADFRIQHPDLILLQYVDDLLLAATSELDCQQGTRALLQTLGNLGYRASAKKAQICQKQVKYLGYLLKEGQRWLTEARKETVMGQPTPKTPRQLREFLGTAGFCRLWIPGFAEMAAPLYPLTKTGTLFNWGPDQQKAYQEIKQALLTAPALGLPDLTKPFELFVDEKQGYAKGVLTQKLGPWRRPVAYLSKKLDPVAAGWPPCLRMVAAIAVLTKDAGKLTMGQPLVILAPHAVEALVKQPPDRWLSNARMTHYQALLLDTDRVQFGPVVALNPATLLPLPEEGLQHNCLDILAEAHGTRPDLTDQPLPDADHTWYTDGSSLLQEGQRKAGAAVTTETEVIWAKALPAGTSAQRAELIALTQALKMAEGKKLNVYTDSRYAFATAHIHGEIYRRRGLLTSEGKEIKNKDEILALLKALFLPKRLSIIHCPGHQKGHSAEARGNRMADQAARKAAITETPDTSTLL

SEQ ID NO: 33 - protein, 667 aa, Unknown
  Feline Leukemia Virus
TLQLEEEYRLFEPESTQKQEMDIWLKNFPQAWAETGGMGMAHCQAPVLIQLKATATPISIRQYPMPHEAYQGIKPHIRRMLDQGILKPCQSPWNTPLLPVKKPGTKDYRPVQDLREVNKRVEDIHPTVPNPYNLLSTLPPSHPWYTVLDLKDAFFCLRLHSESQLLFAFEWRDPEIGLSGQLTWTRLPQGFKNSPTLFDEALHSDLADFRVRYPALVLLQYVDDLLLAAATRTECLEGTKALLETLGNKGYRASAKKAQICLQEVTYLGYSLKDGQRWLTKARKEAILSIPVPKNPRQVREFLGTAGYCRLWIPGFAELAAPLYPLTRPGTLFQWGTEQQLAFENIRKALLSSPALGLPDITKPFELFIDENSGFAKGVLVQKLGPWKRPVAYLSKKLDTVASGWPPCLRMVAAIAILVKDAGKLTLGQPLTILTSHPVEALVRQPPNKWLSNARMTHYQAMLLDAERVHFGPTVSLNPATLLPLPSGKPPRLSPDLAETMAQTDLTDQPLPDADLTWYTDGSSFIRNGERKAGAAVTTESEVIWAASLPPGTSAQRAELIALTQALKMAKGKKLTVYTDSRYAFATAHVHGEIYRRRGLLTSEGKEIKNKNEILALLEALFLPKRLSIIHCPGHQKGDSPQAKGNRLADDTAKKAATETQSSLTIL

SEQ ID NO: 34 - protein, 684 aa, Artificial Sequence
  Synthetic construct
MTLNIEDEYRLHETSKEPDVSLGSTWLSDFPQAWAETGGMGLAVRQAPLIIPLKATSTPVSIKQYPMSQEARLGIKPHIQRLLDQGILVPCQSPWNTPLLPVKKPGTNDYRPVQDLREVNKRVEDIHPTVPNPYNLLSGPPPSHQWYTVLDLKDAFFCLRLHPTSQPLFAFEWRDPEMGISGQLTWTRLPQGFKNSPTLFNEALHRDLADFRIQHPDLILLQYVDDLLLAATSELDCQQGTRALLQTLGNLGYRASAKKAQICQKQVKYLGYLLKEGQRWLTKARKEAILSIPVPKNPRQVREFLGTAGYCRLWIPGFAELAAPLYPLTRPGTLFQWGTEQQLAFENIRKALLSSPALGLPDITKPFELFIDENSGFAKGVLVQKLGPWKRPVAYLSKKLDTVASGWPPCLRMVAAIAILVKDAGKLTLGQPLTILTSHPVEALVRQPPNKWLSNARMTHYQAMLLDAERVHFGPTVSLNPATLLPLPSGKPPRLSPDLAETMAQTDLTDQPLPDADLTWYTAGSSIIRNGERKAGAAVTTESEVIWAASLPPGTSAQRAELIALTQALKMAKGKKLTVYTDSRYAFATAHVHGEIYRRRGLLTSEGKEIKNKNEILALLEALFLPKRLSIIYCPGHQKGDSPQAKGNRLADDTAKKAATETQSSLTILPTELIEGPKRPPWEY

SEQ ID NO: 35 - protein, 684 aa, Artificial Sequence
  Synthetic construct
MTLNIEDEYRLHETSKEPDVSLGSTWLSDFPQAWAETGGMGLAVRQAPLIIPLKATSTPVSIKQYPMSQEARLGIKPHIQRLLDQGILVPCQSPWNTPLLPVKKPGTNDYRPVQDLREVNKRVEDIHPTVPNPYNLLSGPPPSHQWYTVLDLKDAFFCLRLHPTSQPLFAFEWRDPEMGISGQLTWTRLPQGFKNSPTLFNEALHRDLADFRIQHPDLILLQYVDDLLLAAATRTECLEGTKALLETLGNKGYRASAKKAQICLQEVTYLGYSLKDGQRWLTKARKEAILSIPVPKNPRQVREFLGTAGYCRLWIPGFAELAAPLYPLTRPGTLFQWGTEQQLAFENIRKALLSSPALGLPDITKPFELFIDENSGFAKGVLVQKLGPWKRPVAYLSKKLDTVASGWPPCLRMVAAIAILVKDAGKLTLGQPLTILTSHPVEALVRQPPNKWLSNARMTHYQAMLLDAERVHFGPTVSLNPATLLPLPSGKPPRLSPDLAETMAQTDLTDQPLPDADLTWYTGGSSFIRNGERKAGAAVTTESEVIWAASLPPGTSAQRAELIALTQALKMAKGKKLTVYTDSRYAFATAHVHGEIYRRRGWLTSKGKEIKNKNEILALLEALFLPKRLSIIHCPGHQKGDSPQAKGNRLADDTAKKAATETQSSLTILPTELIEGPKRPPWEY

SEQ ID NO: 36 - protein, 278 aa, Artificial Sequence; identical to SEQ ID NO: 4
  Synthetic construct

SEQ ID NO: 37 - protein, 406 aa, Artificial Sequence
  Synthetic construct
RWLTKARKEAILSIPVPKNPRQVREFLGTAGYCRLWIPGFAELAAPLYPLTRPGTLFQWGTEQQLAFENIRKALLSSPALGLPDITKPFELFIDENSGFAKGVLVQKLGPWKRPVAYLSKKLDTVASGWPPCLRMVAAIAILVKDAGKLTLGQPLTILTSHPVEALVRQPPNKWLSNARMTHYQAMLLDAERVHFGPTVSLNPATLLPLPSGKPPRLSPDLAETMAQTDLTDQPLPDADLTWYTAGSSIIRNGERKAGAAVTTESEVIWAASLPPGTSAQRAELIALTQALKMAKGKKLTVYTDSRYAFATAHVHGEIYRRRGLLTSEGKEIKNKNEILALLEALFLPKRLSIIYCPGHQKGDSPQAKGNRLADDTAKKAATETQSSLTILPTELIEGPKRPPWEY

SEQ ID NO: 38 - protein, 222 aa, Artificial Sequence; identical to SEQ ID NO: 3
  Synthetic construct

SEQ ID NO: 39 - protein, 462 aa, Artificial Sequence
  Synthetic construct
YVDDLLLAAATRTECLEGTKALLETLGNKGYRASAKKAQICLQEVTYLGYSLKDGQRWLTKARKEAILSIPVPKNPRQVREFLGTAGYCRLWIPGFAELAAPLYPLTRPGTLFQWGTEQQLAFENIRKALLSSPALGLPDITKPFELFIDENSGFAKGVLVQKLGPWKRPVAYLSKKLDTVASGWPPCLRMVAAIAILVKDAGKLTLGQPLTILTSHPVEALVRQPPNKWLSNARMTHYQAMLLDAERVHFGPTVSLNPATLLPLPSGKPPRLSPDLAETMAQTDLTDQPLPDADLTWYTGGSSFIRNGERKAGAAVTTESEVIWAASLPPGTSAQRAELIALTQALKMAKGKKLTVYTDSRYAFATAHVHGEIYRRRGWLTSKGKEIKNKNEILALLEALFLPKRLSIIHCPGHQKGDSPQAKGNRLADDTAKKAATETQSSLTILPTELIEGPKRPPWEY

SEQ ID NO: 40 - protein, 707 aa, Artificial Sequence
  Synthetic construct
MGSSHHHHHHSSGLVPRGSHMTLNIEDEYRLHETSKEPDVSLGSTWLSDFPQAWAETGGMGLAVRQAPLIIPLKATSTPVSIKQYPMSQEARLGIKPHIQRLLDQGILVPCQSPWNTPLLPVKKPGTNDYRPVQDLREVNKRVEDIHPTVPNPYNLLSGPPPSHQWYTVLDLKDAFFCLRLHPTSQPLFAFEWRDPEMGISGQLTWTRLPQGFKNSPTLFNEALHRDLADFRIQHPDLILLQYVDDLLLAATSELDCQQGTRALLQTLGNLGYRASAKKAQICQKQVKYLGYLLKEGQRWLTKARKEAILSIPVPKNPRQVREFLGTAGYCRLWIPGFAELAAPLYPLTRPGTLFQWGTEQQLAFENIRKALLSSPALGLPDITKPFELFIDENSGFAKGVLVQKLGPWKRPVAYLSKKLDTVASGWPPCLRMVAAIAILVKDAGKLTLGQPLTILTSHPVEALVRQPPNKWLSNARMTHYQAMLLDAERVHFGPTVSLNPATLLPLPSGKPPRLSPDLAETMAQTDLTDQPLPDADLTWYTAGSSIIRNGERKAGAAVTTESEVIWAASLPPGTSAQRAELIALTQALKMAKGKKLTVYTDSRYAFATAHVHGEIYRRRGLLTSEGKEIKNKNEILALLEALFLPKRLSIIYCPGHQKGDSPQAKGNRLADDTAKKAATETQSSLTILPTELIEGPKRPPWEYAAA

SEQ ID NO: 41 - protein, 707 aa, Artificial Sequence
  Synthetic construct
MGSSHHHHHHSSGLVPRGSHMTLNIEDEYRLHETSKEPDVSLGSTWLSDFPQAWAETGGMGLAVRQAPLIIPLKATSTPVSIKQYPMSQEARLGIKPHIQRLLDQGILVPCQSPWNTPLLPVKKPGTNDYRPVQDLREVNKRVEDIHPTVPNPYNLLSGPPPSHQWYTVLDLKDAFFCLRLHPTSQPLFAFEWRDPEMGISGQLTWTRLPQGFKNSPTLFNEALHRDLADFRIQHPDLILLQYVDDLLLAAATRTECLEGTKALLETLGNKGYRASAKKAQICLQEVTYLGYSLKDGQRWLTKARKEAILSIPVPKNPRQVREFLGTAGYCRLWIPGFAELAAPLYPLTRPGTLFQWGTEQQLAFENIRKALLSSPALGLPDITKPFELFIDENSGFAKGVLVQKLGPWKRPVAYLSKKLDTVASGWPPCLRMVAAIAILVKDAGKLTLGQPLTILTSHPVEALVRQPPNKWLSNARMTHYQAMLLDAERVHFGPTVSLNPATLLPLPSGKPPRLSPDLAETMAQTDLTDQPLPDADLTWYTGGSSFIRNGERKAGAAVTTESEVIWAASLPPGTSAQRAELIALTQALKMAKGKKLTVYTDSRYAFATAHVHGEIYRRRGWLTSKGKEIKNKNEILALLEALFLPKRLSIIHCPGHQKGDSPQAKGNRLADDTAKKAATETQSSLTILPTELIEGPKRPPWEYAAA

SEQ ID NO: 42 - protein, 8 aa, Artificial Sequence
  Synthetic construct
DYKDDDDK